European Patent Specification EP 3 416 669 B1, published May 28, 2025. Title: Means and methods for treating bacterial infections. Applicant: Forschungszentrum Borstel Freie Universität Berlin Universität zu Lübeck Rheinisch-Westfälische Technische Hochschule (RWTH) Aachen. The sequence listing filed with the application follows.

SEQUENCE LISTING (2 sequences)

SEQ ID NO: 1 - protein, 19 aa, Artificial Sequence
  Peptide 19-4LF
GKKYRRFRWKFKGKLFLFG

SEQ ID NO: 2 - protein, 20 aa, Artificial Sequence
  Peptide 19-2.5
GCKKYRRFRWKFKGKFWFWG